European Patent Application EP 4 603 111 A1, published August 20, 2025. Title: NOVEL BIOARTIFICIAL VASCULAR GRAFTS AND METHODS FOR THEIR FABRICATION. Applicant: Christian-Albrechts-Universität zu Kiel. Application EP. The sequence listing filed with the application follows.

SEQUENCE LISTING (8 sequences)

SEQ ID NO: 1 - protein, 4 aa, synthetic construct
LGPA

SEQ ID NO: 2 - protein, 5 aa, synthetic construct
  MOD_RES 1: note = X = N-(3-[2-Furyl]acryloyl)-
XLGPA

SEQ ID NO: 3 - protein, 6 aa, synthetic construct
SIKVAV

SEQ ID NO: 4 - protein, 6 aa, synthetic construct
VGVAPG

SEQ ID NO: 5 - protein, 6 aa, synthetic construct
VGVAPG

SEQ ID NO: 6 - protein, 6 aa, synthetic construct
KQAGDV

SEQ ID NO: 7 - protein, 10 aa, synthetic construct
KSIRVAVAPG

SEQ ID NO: 8 - protein, 10 aa, synthetic construct
KSIRVGVGPG